European Patent Application EP 4 324 846 A1, published February 21, 2024. Title: Inhibitor protein of ligands of epidermal growth factor receptor (EGFR). Applicant: Eberhard Karls Universität Tübingen - Medizinische Fakultät. The sequence listing filed with the application follows.

SEQUENCE LISTING (4 sequences)

SEQ ID NO: 1 - protein, 160 aa, synthetic construct
ANGIGIGEFKDSLSIXAWNIKHFKNAXSISGDLHILPVAFRGDSFTHXPPLEPKELEILKTVKEITGYLLXQAWPENRTDLHAFENLEIIRGRTKQHGQFSLAVVSLNVTSLGLRSLKEISDGDVIMSGNKNLKXANXXNWKKXFGTSGQKTKIISNRGE

SEQ ID NO: 2 - protein, 160 aa, synthetic construct
ANGIGIGEFKDSLSINAWNIKHFKNAQSISGDLHILPVAFRGDSFTHMPPLEPKELEILKTVKEITGYLLIQAWPENRTDLHAFENLEIIRGRTKQHGQFSLAVVSLNVTSLGLRSLKEISDGDVIMSGNKNLKWANKWNWKKVFGTSGQKTKIISNRGE

SEQ ID NO: 3 - protein, 160 aa, synthetic construct
ANGIGIGEFKDSLSIWAWNIKHFKNARSISGDLHILPVAFRGDSFTHTPPLEPKELEILKTVKEITGYLLVQAWPENRTDLHAFENLEIIRGRTKQHGQFSLAVVSLNVTSLGLRSLKEISDGDVIMSGNKNLKMANEMNWKKMFGTSGQKTKIISNRGE

SEQ ID NO: 4 - protein, 168 aa, synthetic construct
CNGIGIGEFKDSLSINATNIKHFKNCTSISGDLHILPVAFRGDSFTHTPPLDPQELDILKTVKEITGFLLIQAWPENRTDLHAFENLEIIRGRTKQHGQFSLAVVSLNITSLGLRSLKEISDGDVIISGNKNLCYANTINWKKLFGTSGQKTKIISNRGENSCKATGQ